European Patent Application EP 4 538 389 A2, published April 16, 2025. Title: Linked Target Capture. Applicant: NCAN Genomics, Inc. Application EP 25155777.3, filed February 4, 2025. The sequence listing filed with the application follows.

SEQUENCE LISTING (6 sequences)

SEQ ID NO: 1 - DNA, 12 bp, synthetic construct
  source 1..12: mol_type = other DNA
cctactcgctac

SEQ ID NO: 2 - DNA, 12 bp, synthetic construct
  source 1..12: mol_type = other DNA
atgcgagcctct

SEQ ID NO: 3 - DNA, 12 bp, synthetic construct
  source 1..12: mol_type = other DNA
gcacctcatcca

SEQ ID NO: 4 - DNA, 12 bp, synthetic construct
  source 1..12: mol_type = other DNA
tgcaggatggtg

SEQ ID NO: 5 - DNA, 19 bp, synthetic construct
  source 1..19: mol_type = other DNA
cttcttctgctgcaactga

SEQ ID NO: 6 - DNA, 19 bp, synthetic construct
  source 1..19: mol_type = other DNA
tccctcctatcatggacac